European Patent Specification EP 4 090 378 B1, published March 27, 2024. Title: Immunoglobulin single domain antibodies for delivery of mucosal vaccines. Applicant: Universiteit Gent. The sequence listing filed with the application follows.

SEQUENCE LISTING (21 sequences)

SEQ ID NO: 1 - protein, 10 aa, Artificial sequence
  CDR sequence
GRTISNHAMG

SEQ ID NO: 2 - protein, 10 aa, Artificial sequence
  CDR sequence
GRTFSSNAMG

SEQ ID NO: 3 - protein, 10 aa, Artificial sequence
  CDR sequence
AISWTGLTTN

SEQ ID NO: 4 - protein, 15 aa, Artificial sequence
  CDR sequence
RQSGYVSKFVDDYGY

SEQ ID NO: 5 - protein, 15 aa, Artificial sequence
  CDR sequence
RQSGYASKFLDEYGY

SEQ ID NO: 6 - protein, 124 aa, Artificial sequence
  Single domain antibody
QVQLQESGGGLVQPGGSLRLSCAGSGRTISNHAMGWFRQAPGKEREFVAAISWTGLTTNYADSVKGRFFISRDDAENTVYLQMNSLKPEDTAVYYCAARQSGYVSKFVDDYGYWGQGTQVTVSS

SEQ ID NO: 7 - protein, 124 aa, Artificial sequence
  Single domain antibody
QVQLQESGGGLVQAGDSLRLSCAGSGRTISNHAMGWFRQAPGKEREFVAAISWTGLTTNYADSVKGRFFISRDDAENTVYLQMNSLEPEDTAVYYCAARQSGYVSKFVDDYGYWGQGTQVTVSS

SEQ ID NO: 8 - protein, 124 aa, Artificial sequence
  Single domain antibody
QVQLQESGGGLVQAGGSLRLSCAASGRTFSSNAMGWFRQAPGKEREFVAAISWTGLTTNYADSVKGRFFISRDDAKNTVYLQMNSLKPEDTAVYYCAARQSGYASKFLDEYGYWGQGTQVTVSS

SEQ ID NO: 9 - protein, 126 aa, Artificial sequence
  Single domain antibody
QVQLQESGGGLVQPGDSLRLSCAASGRTFSTYAMGWFRQAPGKEREFVAYISQLSLSTKYADSVKGRFTVSRDDAQNTLYLQMNSLRPEDTAVYYCATRSQNYVTTYDQSRAYDYWGQGTQVTVSS

SEQ ID NO: 10 - DNA, 432 bp, Artificial sequence
  Single domain antibody
caggtgcagctgcaggagtctgggggaggcttggtgcagcctggggggtctctgagactctcctgtgcaggctctggacgcactattagcaaccatgccatgggctggttccgccaggctccagggaaggagcgcgagtttgtagcagctattagctggactggacttaccacgaactatgcagactccgtgaagggccgattcttcatctccagagacgacgccgagaacacggtgtatctgcaaatgaacagcctgaaacctgaagacacggccgtttattactgtgcagcccgccagtccggttacgtgtcgaaattcgtcgatgactatggctactggggccaggggacccaggtcaccgtctcctcagcggccgcatacccgtacgacgttccggactacggttcccaccaccatcaccatcactag

SEQ ID NO: 11 - DNA, 432 bp, Artificial sequence
  Single domain antibody
caggtgcagctgcaggagtctgggggaggattggtgcaggctggggactctctgagactctcctgtgcaggctctggacgcactattagcaaccatgccatgggctggttccgccaggctccagggaaggagcgcgagtttgtagcagctattagctggactggacttaccacgaactatgcagactccgtgaagggccgattcttcatctccagagacgacgccgagaacacggtgtatctgcaaatgaacagcctggaacctgaagacacggccgtttattactgtgcagcccgccagtccggttacgtgtcgaaattcgtcgatgactatggctactggggccaggggacccaggtcaccgtctcctcagcggccgcatacccgtacgacgttccggactacggttcccaccaccatcaccatcactag

SEQ ID NO: 12 - DNA, 432 bp, Artificial sequence
  Single domain antibody
caggtgcagctgcaggagtctgggggaggattggtgcaggctgggggctctctgagactctcctgcgcagcctctggacgcaccttcagtagtaatgccatgggctggttccgccaggctccagggaaggagcgcgagtttgtagcagctattagctggactggacttaccacgaactatgcagactccgtgaagggccgattcttcatctccagagacgacgccaagaacacggtgtatctgcaaatgaacagcctgaaacctgaagacacggccgtttattactgtgcagcccgccagtccggttacgcgtcgaaattcctcgatgagtatggctactggggccaggggacccaggtcaccgtctcctcagcggccgcatacccgtacgacgttccggactacggttcccaccaccatcaccatcactag

SEQ ID NO: 13 - DNA, 438 bp, Artificial sequence
  Single domain antibody
caggtgcagctgcaggagtctgggggaggattggtgtagcctggggactctctgagactctcctgtgcagcctctggacgcaccttcagtacctatgccatgggctggttccgccaggctccagggaaggagcgtgagtttgtagcctatattagtcaacttagtttgagcacaaagtatgcagactccgtgaagggccgattcaccgtctccagagacgacgcccagaacacgctgtatctgcagatgaacagtctgagacctgaggacacggccgtgtattactgtgccactaggagccaaaattatgttactacttacgatcagtccagggcgtatgactactggggccaggggacccaggtcaccgtctcctcagcggccgcatacccgtacgacgttccggactacggttcccaccaccatcaccatcactag

SEQ ID NO: 14 - protein, 10 aa, Artificial sequence
  CDR sequence
GRTFSTYAMG

SEQ ID NO: 15 - protein, 10 aa, Artificial sequence
  CDR sequence
YISQLSLSTK

SEQ ID NO: 16 - protein, 17 aa, Artificial sequence
  CDR sequence
RSQNYVTTYDQSRAYDY

SEQ ID NO: 17 - protein, 357 aa, Artificial sequence
  VHH-MG fusion
QVQLQESGGGLVQPGGSLRLSCAGSGRTISNHAMGWFRQAPGKEREFVAAISWTGLTTNYADSVKGRFFISRDDAENTVYLQMNSLKPEDTAVYYCAARQSGYVSKFVDDYGYWGQGTQVTVSSEPRGPTIKPCPPCKCPAPNLLGGPSVFIFPPKIKDVLMISLSPIVTCVVVDVSEDDPDVQISWFVNNVEVHTAQTQTHREDYNSTLRVVSALPIQHQDWMSGKEFKCKVNNKDLPAPIERTISKPKGSVRAPQVYVLPPPEEEMTKKQVTLTCMVTDFMPEDIYVEWTNNGKTELNYKNTEPVLDSDGSYFMYSKLRVEKKNWVERNSYSCSVVHEGLHNHHTTKSFSRTPGK

SEQ ID NO: 18 - protein, 342 aa, Artificial sequence
  porcine Fc domain
VSETSPKIFPLTLGSSEPAGYVVIACLVRDFFPSEPLTVTWSPSREGVIVRNFPPAQAGGLYTMSSQLTLPVEQCPADQILKCQVQHLSKSSQSVNVPCKVLPSDPCPQCCKPSLSLQPPALADLLLGSNASLTCTLSGLKKSEGVSFTWQPSGGKDAVQASPTRDSCGCYSVSSILPGCADPWNKGETFSCTAAHSELKSALTATITKPKVNTFRPQVHLLPPPSEELALNELVTLTCLVRGFSPKDVLVRWLQGGQELPRDKYLVWESLPEPGQAIPTYAVTSVLRVDAEDWKQGDTFSCMVGHEALPLAFTQKTIDRLAGKPTHVNVSVVMAEAEGICY

SEQ ID NO: 19 - protein, 238 aa, Artificial sequence
  porcine Fc domain
DPCPQCCKPSLSLQPPALADLLLGSNASLTCTLSGLKKSEGVSFTWQPSGGKDAVQASPTRDSCGCYSVSSILPGCADPWNKGETFSCTAAHSELKSALTATITKPKVNTFRPQVHLLPPPSEELALNELVTLTCLVRGFSPKDVLVRWLQGGQELPRDKYLVWESLPEPGQAIPTYAVTSVLRVDAEDWKQGDTFSCMVGHEALPLAFTQKTIDRLAGKPTHVNVSVVMAEAEGICY

SEQ ID NO: 20 - protein, 333 aa, Artificial sequence
  porcine Fc domain
AYNTAPSVYPLAPCGRDVSDHNVALGCLVSSYFPEPVTVTWNSGALSRVVHTFPSVLQPSGLYSLSSMVIVAASSLSTLSYTCNVYHPATNTKVDKRVDIEPPTPICPEICSCPAAEVLGAPSVFLFPPKPKDILMISRTPKVTCVVVDVSQEEAEVQFSWYVDGVQLYTAQTRPMEEQFNSTYRVVSVLPIQHQDWLKGKEFKCKVNNKDLLSPITRTISKATGPSRVPQVYTLPPAWEELSKSKVSITCLVTGFYPPDIDVEWQSNGQQEPEGNYRTTPPQQDVDGTYFLYSKLAVDKVRWQRGDLFQCAVMHEALHNHYTQKSISKTQGK

SEQ ID NO: 21 - protein, 329 aa, Artificial sequence
  porcine Fc domain
APSVYPLAPCGRDVSDHNVALGCLVSSYFPEPVTVTWNSGALSRVVHTFPSVLQPSGLYSLSSMVIVAASSLSTLSYTCNVYHPATNTKVDKRVDIEPPTPICPEICSCPAAEVLGAPSVFLFPPKPKDILMISRTPKVTCVVVDVSQEEAEVQFSWYVDGVQLYTAQTRPMEEQFNSTYRVVSVLPIQHQDWLKGKEFKCKVNNKDLLSPITRTISKATGPSRVPQVYTLPPAWEELSKSKVSITCLVTGFYPPDIDVEWQSNGQQEPEGNYRTTPPQQDVDGTYFLYSKLAVDKVRWQRGDLFQCAVMHEALHNHYTQKSISKTQGK